European Patent Specification EP 3 630 954 B1, published August 9, 2023. Title: METHOD FOR EXPANDING STEMNESS AND DIFFERENTIATION POTENTIAL OF PLURIPOTENT CELLS. Applicant: Fundación Centro Nacional de Investigaciones Oncológicas Carlos III. The sequence listing filed with the application follows.

SEQUENCE LISTING (86 sequences)

SEQ ID NO: 1 - RNA, 22 nt, Homo sapiens
  misc_feature (1)..(22): hsa-miR203a-3p: Accession MIMAT0000264 in miRBase
  misc_feature (2)..(8): Seed region
gugaaauguuuaggaccacuag

SEQ ID NO: 2 - RNA, 110 nt, Homo sapiens
  misc_feature (1)..(110): hsa-miR203a, Accession MI0000283 in miRBase
guguuggggacucgcgcgcuggguccagugguucuuaacaguucaacaguucuguagcgcaauugugaaauguuuaggaccacuagacccggcgggcgcggcgacagcga

SEQ ID NO: 3 - RNA, 76 nt, Mus musculus
  misc_features (1)..(76): mmu-miR-203, Accession MI0000246 in miRBase
gccugguccagugguucuugacaguucaacaguucuguagcacaauugugaaauguuuaggaccacuagacccggc

SEQ ID NO: 4 - RNA, 22 nt, Mus musculus
  misc_feature (1)..(22): mmu-miR-203-3p: Accession MIMAT0000236 in miRbase
gugaaauguuuaggaccacuag

SEQ ID NO: 5 - DNA, 21 bp, Artificial sequence
  Forward primer of RT-PCR of mouse gene Dazl
ggttttaccacccgaactctg

SEQ ID NO: 6 - DNA, 21 bp, Artificial sequence
  Reverse primer of RT-PCR of mouse gene Dazl
tgtggttgctgatgaagactg

SEQ ID NO: 7 - DNA, 20 bp, Artificial sequence
  Forward primer of RT-PCR of mouse gene Dnmt1
cagagactcccgaggacaga

SEQ ID NO: 8 - DNA, 22 bp, Artificial sequence
  Reverse primer of RT-PCR of mouse gene Dnmt1
tttacgtgtcgtttttcgtctc

SEQ ID NO: 9 - DNA, 19 bp, Artificial sequence
  Forward primer of RT-PCR of mouse gene Dnmt3a
aaacggaaacgggatgagt

SEQ ID NO: 10 - DNA, 22 bp, Artificial sequence
  Reverse primer of RT-PCR of mouse gene Dnmt3a
actgcaattaccttggctttct

SEQ ID NO: 11 - DNA, 22 bp, Artificial sequence
  Forward primer of RT-PCR of mouse gene Dnmt3a2
gggcaaactgaagtagtgatga

SEQ ID NO: 12 - DNA, 18 bp, Artificial sequence
  Reverse primer of RT-PCR of mouse gene Dnmt3a2
ttacacggcacctgctga

SEQ ID NO: 13 - DNA, 18 bp, Artificial sequence
  Forward primer of RT-PCR of mouse gene Dnmt3b
ccctcccccatccatagt

SEQ ID NO: 14 - DNA, 21 bp, Artificial sequence
  Reverse primer of RT-PCR of mouse gene Dnmt3b
tctgctgtctcccttcattgt

SEQ ID NO: 15 - DNA, 19 bp, Artificial sequence
  Forward primer of RT-PCR of mouse gene Dnmt3l
aagtgaaccgacggagcat

SEQ ID NO: 16 - DNA, 22 bp, Artificial sequence
  Reverse primer of RT-PCR of mouse gene Dnmt3l
ccgagtgtacacctggagagtt

SEQ ID NO: 17 - DNA, 28 bp, Artificial sequence
  Forward primer of RT-PCR of mouse gene Ecat1
tgtggggccctgaaaggcgagctgagat

SEQ ID NO: 18 - DNA, 28 bp, Artificial sequence
  Reverse primer of RT-PCR of mouse gene Ecat1
atgggccgccatacgacgacgctcaact

SEQ ID NO: 19 - DNA, 24 bp, Artificial sequence
  Forward primer of RT-PCR of mouse gene Eras
actgcccctcatcagactgctact

SEQ ID NO: 20 - DNA, 24 bp, Artificial sequence
  Reverse primer of RT-PCR of mouse gene Eras
cactgccttgtactcgggtagctg

SEQ ID NO: 21 - DNA, 24 bp, Artificial sequence
  Forward primer of RT-PCR of mouse gene Esg1
gaagtctggttccttggcaggatg

SEQ ID NO: 22 - DNA, 20 bp, Artificial sequence
  Reverse primer of RT-PCR of mouse gene Esg1
actcgatacactggcctagc

SEQ ID NO: 23 - DNA, 23 bp, Artificial sequence
  Forward primer of RT-PCR of mouse gene Fgf4
cgtggtgagcatcttcggagtgg

SEQ ID NO: 24 - DNA, 23 bp, Artificial sequence
  Reverse primer of RT-PCR of mouse gene Fgf4
ccttcttggtccgcccgttctta

SEQ ID NO: 25 - DNA, 21 bp, Artificial sequence
  Forward primer of RT-PCR of mouse gene Gapdh
aggtcggtgtgaacggatttg

SEQ ID NO: 26 - DNA, 23 bp, Artificial sequence
  Reverse primer of RT-PCR of mouse gene Gapdh
tgtagaccatgtagttgaggtca

SEQ ID NO: 27 - DNA, 28 bp, Artificial sequence
  Forward primer of RT-PCR of mouse gene Gata6
accttatggcgtagaaatgctgagggtg

SEQ ID NO: 28 - DNA, 28 bp, Artificial sequence
  Reverse primer of RT-PCR of mouse gene Gata6
ctgaatacttgaggtcactgttctcggg

SEQ ID NO: 29 - DNA, 24 bp, Artificial sequence
  Forward primer of RT-PCR of mouse gene Gdf3
gttccaacctgtgcctcgcgtctt

SEQ ID NO: 30 - DNA, 26 bp, Artificial sequence
  Reverse primer of RT-PCR of mouse gene Gdf3
agcgaggcatggagagagcggagcag

SEQ ID NO: 31 - DNA, 21 bp, Artificial sequence
  Forward primer of RT-PCR of mouse gene Hcn1
tgaagctgacagatggctctt

SEQ ID NO: 32 - DNA, 20 bp, Artificial sequence
  Reverse primer of RT-PCR of mouse gene Hcn1
ctggcagtacgacgtccttt

SEQ ID NO: 33 - DNA, 24 bp, Artificial sequence
  Forward primer of RT-PCR of mouse gene Isl1
ttgtacgggatcaaatgcgccaag

SEQ ID NO: 34 - DNA, 19 bp, Artificial sequence
  Reverse primer of RT-PCR of mouse gene Isl1
aggccacacagcggaaaca

SEQ ID NO: 35 - DNA, 20 bp, Artificial sequence
  Forward primer of RT-PCR of mouse gene Kcna4
tcattgctctgacctgatgc

SEQ ID NO: 36 - DNA, 20 bp, Artificial sequence
  Reverse primer of RT-PCR of mouse gene Kcna4
tcactcagctccctcaggat

SEQ ID NO: 37 - DNA, 20 bp, Artificial sequence
  Forward primer of RT-PCR of mouse gene Kcnh2
acgcttactgccagggtgac

SEQ ID NO: 38 - DNA, 18 bp, Artificial sequence
  Reverse primer of RT-PCR of mouse gene Kcnh2
gccgactggcaaccagag

SEQ ID NO: 39 - DNA, 20 bp, Artificial sequence
  Forward primer of RT-PCR of mouse gene Myh
ctcaagctcatggccactct

SEQ ID NO: 40 - DNA, 21 bp, Artificial sequence
  Reverse primer of RT-PCR of mouse gene Myh
gcctcctttgcttttaccact

SEQ ID NO: 41 - DNA, 20 bp, Artificial sequence
  Forward primer of RT-PCR of mouse gene Nanog
caggtgtttgagggtagctc

SEQ ID NO: 42 - DNA, 20 bp, Artificial sequence
  Reverse primer of RT-PCR of mouse gene Nanog
cggttcatcatggtacagtc

SEQ ID NO: 43 - DNA, 22 bp, Artificial sequence
  Forward primer of RT-PCR of mouse gene Nppa
gaaccagaggggagagacagag

SEQ ID NO: 44 - DNA, 22 bp, Artificial sequence
  Reverse primer of RT-PCR of mouse gene Nppa
ccctcagcttgctttttaggag

SEQ ID NO: 45 - DNA, 26 bp, Artificial sequence
  Forward primer of RT-PCR of mouse gene Tbx5
aaatgaaacccagcataggagctggc

SEQ ID NO: 46 - DNA, 24 bp, Artificial sequence
  Reverse primer of RT-PCR of mouse gene Tbx5
acactcagcctcacatcttaccct

SEQ ID NO: 47 - DNA, 22 bp, Artificial sequence
  Forward primer of RT-PCR of mouse gene Tnnt2
ggcagcggaagaggatgctgaa

SEQ ID NO: 48 - DNA, 25 bp, Artificial sequence
  Reverse primer of RT-PCR of mouse gene Tnnt2
gaggcaccaagttgggcatgaacga

SEQ ID NO: 49 - RNA, 17 nt, Mus musculus
  3'UTR (1)..(17): Fragment of 3'UTR Dnmt3a
  misc_feature (10)..(16): Seed region of miR-203
aauaauguacauuucac

SEQ ID NO: 50 - RNA, 17 nt, Artificial sequence
  Mutated version of 3'-UTR of Dnmt3a of Mus musculus
  mutation (11)..(11): A replaced by C with regard to the natural sequence of Dnmt3a mRNA 3' UTR
  mutation (13)..(13): U replaced by A with regard to the natural sequence of Dnmt3a mRNA 3' UTR
  mutation (15)..(15): C replaced by A with regard to the natural sequence of Dnmt3a mRNA 3' UTR
aauaauguaccuauaac

SEQ ID NO: 51 - RNA, 17 nt, Mus musculus
  3'UTR (1)..(17): 3'UTR of Dnmt3b
  misc_feature (9)..(15): Seed region of miR-203
gaaagcugcauuucaga

SEQ ID NO: 52 - RNA, 17 nt, Artificial sequence
  Mutated version of 3'UTR of Dnmtb
  mutation (10)..(10): A replaced by C with regard to the natural sequence of Dnmtb mRNA 3' UTR
  mutation (12)..(12): U replaced by A with regard to the natural sequence of Dnmtb mRNA 3' UTR
  mutation (14)..(14): C replaced by A with regard to the natural sequence of Dnmtb mRNA 3' UTR
gaaagcugccuauaaga

SEQ ID NO: 53 - RNA, 25 nt, Homo sapiens
  misc_feature (1)..(25): hsa-miR203a-5p: Accession MIMAT0031890 in miRBase
  misc_feature (11)..(11): a is replaced by g in mmu-miR203-5p
  misc_feature (23)..(25): nucleotides absent from mmu-mi203-5p
agugguucuuaacaguucaacaguu

SEQ ID NO: 54 - RNA, 22 nt, Mus musculus
  misc_feature (1)..(22): mmu-miR-203-5p, Accession MIMAT0004547 in miRBase
  misc_feature (11)..(11): g is replaced by a in hsa-miR203a-5p
agugguucuugacaguucaaca

SEQ ID NO: 55 - DNA, 28 bp, Artificial sequence
  Primer Dnmt3a EcoRI-Fw for PCR amplificacion of Dnmt3a
gaattcagggacatgggggcaaactgaa

SEQ ID NO: 56 - DNA, 30 bp, Artificial sequence
  Primer Dnmt3a EcoRI-Rv for PCR amplificacion of Dnmt3a
catatgctgaggcagtcattttagattcat

SEQ ID NO: 57 - DNA, 27 bp, Artificial sequence
  Primer Dnmt3b_EcoRI-Fw for PCR amplification of Dnmt3b
gaattcttttagctcacctgtgtgggg

SEQ ID NO: 58 - DNA, 28 bp, Artificial sequence
  Primer Dnmt3b_NdeI-Rv for PCR amplification of Dnmt3b
catatgccagaaaggtaaactctgggca

SEQ ID NO: 59 - DNA, 31 bp, Artificial sequence
  Primer Dnmt31_EcoRI-Fw for PCR amplification of Dnmt31
gaattcgaaatgaatcaccataagatgaaag

SEQ ID NO: 60 - DNA, 32 bp, Artificial sequence
  Primer Dnmt31_NdeI-Rv for PCR amplification of Dnmt31
catatgaacaatcctatgatatatttgaaaaa

SEQ ID NO: 61 - DNA, 27 bp, Artificial sequence
  Primer Dnmt1_NdeI-Rv for PCR amplification of Dnmt1
gaattcgtgctctcacccagagcccca

SEQ ID NO: 62 - DNA, 30 bp, Artificial sequence
  Primer Dnmt1_NdeI-Rv for PCR amplification of Dnmt1
catatggcttgacagaagcgctttattttg

SEQ ID NO: 63 - DNA, 28 bp, Artificial sequence
  Forward primer of RT-PCR of mouse gene Ecat1
tgtggggccctgaaaggcgagctgagat

SEQ ID NO: 64 - DNA, 28 bp, Artificial sequence
  Reverse primer of RT-PCR of mouse gene Ecat1
atgggccgccatacgacgacgctcaact

SEQ ID NO: 65 - DNA, 24 bp, Artificial sequence
  Forward primer of RT-PCR of mouse gene Eras
actgcccctcatcagactgctact

SEQ ID NO: 66 - DNA, 24 bp, Artificial sequence
  Reverse primer of RT-PCR of mouse gene Eras
cactgccttgtactcgggtagctg

SEQ ID NO: 67 - DNA, 24 bp, Artificial sequence
  Forward primer of RT-PCR of mouse gene Esg1
gaagtctggttccttggcaggatg

SEQ ID NO: 68 - DNA, 20 bp, Artificial sequence
  Reverse primer of RT-PCR of mouse gene Esg1
actcgatacactggcctagc

SEQ ID NO: 69 - DNA, 23 bp, Artificial sequence
  Forward primer of RT-PCR of mouse gene Fgf4
cgtggtgagcatcttcggagtgg

SEQ ID NO: 70 - DNA, 23 bp, Artificial sequence
  Reverse primer of RT-PCR of mouse gene Fgf4
ccttcttggtccgcccgttctta

SEQ ID NO: 71 - DNA, 24 bp, Artificial sequence
  Forward primer of RT-PCR of mouse gene Gdf3
gttccaacctgtgcctcgcgtctt

SEQ ID NO: 72 - DNA, 26 bp, Artificial sequence
  Reverse primer of RT-PCR of mouse gene Gdf3
agcgaggcatggagagagcggagcag

SEQ ID NO: 73 - DNA, 25 bp, Artificial sequence
  Forward primer of RT-PCR of rat gene Ccnb1
ggagatgaagattctgagagttctg

SEQ ID NO: 74 - DNA, 20 bp, Artificial sequence
  Reverse primer of RT-PCR of rat gene Ccnb1
gtatgctgctccacatcgac

SEQ ID NO: 75 - DNA, 20 bp, Artificial sequence
  Forward primer of RT-PCR of rat gene Gapdh
ggcaagttcaatggcacagt

SEQ ID NO: 76 - DNA, 22 bp, Artificial sequence
  Reverse primer of RT-PCR of rat gene Gapdh
tggtgaagacgccagtagactc

SEQ ID NO: 77 - DNA, 18 bp, Artificial sequence
  Forward primer of RT-PCR of rat gene Myh6
gggctggagcactgagag

SEQ ID NO: 78 - DNA, 20 bp, Artificial sequence
  Reverse primer of RT-PCR of rat gene Myh6
gagagaggaacaggcaggaa

SEQ ID NO: 79 - DNA, 18 bp, Artificial sequence
  Forward primer of RT-PCR of rat gene Myh7
atggcggatcgagagatg

SEQ ID NO: 80 - DNA, 18 bp, Artificial sequence
  Reverse primer of RT-PCR of rat gene Myh7
ggtcaaagggcctggtct

SEQ ID NO: 81 - DNA, 29 bp, Artificial sequence
  Forward primer for DNA mehylation analysis of mouse gene Elf5 (a)
taaaggttgtaatgaatagatattaggtt

SEQ ID NO: 82 - DNA, 32 bp, Artificial sequence
  Reverse primer for DNA mehylation analysis of mouse gene Elf5 (a)
aactacttacttaaaaacaaataataactaaa

SEQ ID NO: 83 - DNA, 29 bp, Artificial sequence
  Forward primer for DNA mehylation analysis of mouse gene Elf5 (b)
taaaggttgtaatgaatagatattaggtt

SEQ ID NO: 84 - DNA, 27 bp, Artificial sequence
  Reverse primer for DNA mehylation analysis of mouse gene Elf5 (b)
aaataataactaaatccaaacaaaaaa

SEQ ID NO: 85 - DNA, 30 bp, Artificial sequence
  Forward primer for DNA mehylation analysis of mouse gene Sirt6
tttggttttttttaggttatgttaggattt

SEQ ID NO: 86 - DNA, 27 bp, Artificial sequence
  Reverse primer for DNA mehylation analysis of mouse gene Sirt6
cacttacctctacctcccaataaaaaa